European Patent Application EP 4 592 679 A1, published July 30, 2025. Title: USE OF DISCOIDIN DOMAIN RECEPTOR 2 IN DIAGNOSIS OF NEURODEGENERATIVE DISEASES, AND RELATED COMPUTER READABLE MEDIUM. Applicant: FIBROINOVA BIOMEDICAL TECHNOLOGY (GUANGZHOU) COMPANY, LTD. The sequence listing filed with the application follows.

SEQUENCE LISTING (4 sequences)

SEQ ID NO: 1 - protein, 8 aa, synthetic construct
GYILSPNV

SEQ ID NO: 2 - protein, 8 aa, synthetic construct
ISWGDGRT

SEQ ID NO: 3 - protein, 17 aa, synthetic construct
AASRKGYPSTRSDPYNY

SEQ ID NO: 4 - protein, 124 aa, synthetic construct
EVQLVESGGGLVQPGGSLRLSCAASGYILSPNVMGWFRQAPGKGRELVAAISWGDGRTYYPDSVEGRFTISRDNAKRMVYLQMNSLRAEDTAVYYCAASRKGYPSTRSDPYNYWGQGTQVTVSS